European Patent Specification EP 3 218 005 B1, published January 4, 2023. Title: GLYCAN-INTERACTING COMPOUNDS AND METHODS OF USE. Applicant: SIAMAB THERAPEUTICS, INC. The sequence listing filed with the application follows.

SEQUENCE LISTING (244 sequences)

SEQ ID NO: 1 - protein, 121 aa, Artificial Sequence
  Description of Artificial Sequence: Synthetic polypeptide
QVTLKESGPGILQPSQTLSLTCSFSGFSLSTSNMGIGWIRQPSGKGLEWLAHIWWHDDKYYNPSLKSRLTISKDISNNQVFLKITSVDTADTATYYCAQVPFYYGTSFDVWGTGTTVTVSS

SEQ ID NO: 2 - protein, 107 aa, Artificial Sequence
  Description of Artificial Sequence: Synthetic polypeptide
DIVMTQSPATLSVTPGDRVSLSCRASQSISDYLHWYQQKSHESPRLLIKYASQSISGIPSRFSGSGSGSDFTLSINSVEPEDVGVYYCQNGHSFPLTFGAGTKLELK

SEQ ID NO: 3 - protein, 105 aa, Artificial Sequence
  Description of Artificial Sequence: Synthetic polypeptide
QIVLTQSPAIMSASPGETVTMTCSASSSITYMHWYQQKPGTSPKRWIYDTSKLASGVPARFSGSGSGTSYSLTISSMEAEDAATYYCHQRSSYTFGGGTKLEIKR

SEQ ID NO: 4 - protein, 121 aa, Artificial Sequence
  Description of Artificial Sequence: Synthetic polypeptide
QVTLKESGPGILQPSQTLSLTCSFSGFSLSTFGMGVGWIRQPSGKGLEWLAHIWWDDDKYYNPALKSRLTISKDTSKNQVFLKIANVDTADTATYYCARIAYYYGSERDYWGQGTTLTVSS

SEQ ID NO: 5 - protein, 105 aa, Artificial Sequence
  Description of Artificial Sequence: Synthetic polypeptide
QIVLTQSPAIMSASPGEKVTMTCSASSSISYMHWYHQKPGTSPKRWIYDTSKLASGVPARFSGSGSGTSYSLTISSMEAEDAATYYCHQRSSYTFGGGTKLEIKR

SEQ ID NO: 6 - protein, 112 aa, Artificial Sequence
  Description of Artificial Sequence: Synthetic polypeptide
QVQLKESGPGLVAPSQSLSITCTVSGFSLTSYGVSWVRQPPGKGLEWLGVIWGDGSTNYHSSLISRLSISKDNSKSQVFLKLNSLQTDDTATYYCARAFVYWGQGTLVTVSA

SEQ ID NO: 7 - protein, 108 aa, Artificial Sequence
  Description of Artificial Sequence: Synthetic polypeptide
QIVLTQSPAIMSASPGEKVTMTCSASSSVSYIHWYQQKSGTSPKRWIYDTSKLASGVPARFSGSGSGTSYSLTISSMEAEDAATYYCQQWSSNPPMLTFGAGTKLELK

SEQ ID NO: 8 - protein, 112 aa, Artificial Sequence
  Description of Artificial Sequence: Synthetic polypeptide
QVQLKESGPGLVAPSQSLSITCTVSGFSLTSYGVSWVRQPPGKGLEWLGVIWGDGSTNYHSALISRLIISKDNSKSQVFLKLNSLQTDDTATYYCTKGFTYWGQGTLVTVSA

SEQ ID NO: 9 - protein, 106 aa, Artificial Sequence
  Description of Artificial Sequence: Synthetic polypeptide
QIVLTQSPAIMSASPGEKVTMTCSASSSVSYMHWYQQKSGTSPKRWIFDTSKLASGVPARFSGSGSGTSYSLTISSMEAEDAATYYCQQWSSNLLTFGAGTKLELK

SEQ ID NO: 10 - protein, 112 aa, Artificial Sequence
  Description of Artificial Sequence: Synthetic polypeptide
QVQLQESGPGLVAPSQSLSITCTVSGFSLISYGVNWVRQPPGKGLEWLGVIWGDGSTNYQSALISRLIISKDNSKSQVFLKLNSLQTDDTATYYCTKGFAYWGQGTLVTVSA

SEQ ID NO: 11 - protein, 106 aa, Artificial Sequence
  Description of Artificial Sequence: Synthetic polypeptide
QIVLTQSPAIMSASPGEKVTMTCSASSSVSYMHWFQQKSGTSPKRWIYDTSKLASGVPARFSGSGSGTSYSLTISSMEAEDAATYYCQQWSSNLLTFGAGTKLELK

SEQ ID NO: 12 - protein, 112 aa, Artificial Sequence
  Description of Artificial Sequence: Synthetic polypeptide
QVQLKESGPGLVAPSQNLSITCTVSGFSLTSYGVNWVRQPPGKGLEWLGVIWGDGSTNYHSALISRLIISKENSKSQVFLKLNSLQTNDTATYYCTKGFVYWGQGTLVTVSA

SEQ ID NO: 13 - protein, 114 aa, Artificial Sequence
  Description of Artificial Sequence: Synthetic polypeptide
QVQLKESGPGLVAPSQSLSITCTVSGFSLTSYGVSWVRQPPGKGLEWLGVIWGDGSTNYHSALISRLSISKDNSKSQVFLKLNSLQTDDTATYYCAKGGYFDYWGQGTTLTVSS

SEQ ID NO: 14 - protein, 106 aa, Artificial Sequence
  Description of Artificial Sequence: Synthetic polypeptide
QIVLTQSPAVMSASPGEKVAITCSASSSVSYMHWFQQKPGTSPKLWIYSTSNLASGVPARFSGSGSGTSYSLTISRMEAEDAATYYCQQRSSYPWTFGGGTKLEIK

SEQ ID NO: 15 - protein, 115 aa, Artificial Sequence
  Description of Artificial Sequence: Synthetic polypeptide
QVQLLQYDAELVKPGGSVKISCKASGYTFTDHAIHWVKQKPEQGLEWIGYFSPGNDDIKYSEKFKGKATLTADKSSSTAYMQLNSLTSEDSAVYFCKRSITTPYWGQGTLVTVSA

SEQ ID NO: 16 - protein, 106 aa, Artificial Sequence
  Description of Artificial Sequence: Synthetic polypeptide
DIQMNQSPSSLSASLGDTITITCHASQNINVWLSWYQQKPGNIPKLLIYKVSNLHTGVPSRFSGSGSGTGFTLTISSLQPEDIATYYCQQDQSYPYTFGGGTKLKK

SEQ ID NO: 17 - protein, 115 aa, Artificial Sequence
  Description of Artificial Sequence: Synthetic polypeptide
QVQLQQSDAELVKPGASVKISCKASGYTFTDHAIHWVKQKPEQGLEWIGYISPGNDDIKYNEKFKGKATLTADKSSSTAYMQLNSLTSEDSAVYFCKRSITTSYWGQGTLVTVSA

SEQ ID NO: 18 - protein, 108 aa, Artificial Sequence
  Description of Artificial Sequence: Synthetic polypeptide
NIVMTQSPKSMSMSVGERVTLTCKASENVVIYVSWYQQKPEQSPKLLIYGASNRYTGVPDRFTGSGSATDFTLTISSVQAEDLADYHCGQGYSYPYTFGGGTKLEIKR

SEQ ID NO: 19 - protein, 115 aa, Artificial Sequence
  Description of Artificial Sequence: Synthetic polypeptide
QVQLQQSDAELVKPGASVKISCKASGYTFTDHAIHWVKQKPEQGLEWIGYVSPGNGDIKYNEKFKGKATLTADKSSSTAYMQLNSLTSEDSAVYFCKRSLIGDYWGQGTTLTVSS

SEQ ID NO: 20 - protein, 107 aa, Artificial Sequence
  Description of Artificial Sequence: Synthetic polypeptide
DIVMTQSQKFMSSSVGDRVTITCKASQNVGTAVAWYQQKPGQSPKFLIYSASNRYTGVPDRFTGSGSGTDFTLTISNMQSEDLADYFCQQYSSYRLTFGGGTKLEIK

SEQ ID NO: 21 - protein, 115 aa, Artificial Sequence
  Description of Artificial Sequence: Synthetic polypeptide
QVQLQQSDAELVKPGASVKISCKASGYTFTDHAIHWVKQKPEQGLEWIGYLSPGNDDIKYSEKFKDKATLTADKSSSTAYMQLNSLTSEDSAVYFCKRSIGGDHWGQGTTLTVSS

SEQ ID NO: 22 - protein, 108 aa, Artificial Sequence
  Description of Artificial Sequence: Synthetic polypeptide
DIQMNQSPSSLSASLGDTITITCHASQNINVWLNWYQQKPGNIPKLLIYKASNLHTGVPSRFSGSGSGTGFTLTIGSLQPEDIATYYCQQGQSYPFTFGGGTKLEIKR

SEQ ID NO: 23 - protein, 115 aa, Artificial Sequence
  Description of Artificial Sequence: Synthetic polypeptide
QVQLQQSDAELVKPGASVKISCKASGYTFTDHAIHWVKQKPEQGLEWIGYISPGNGDIKYNEKFKGKATLTADKSSSTAYMQLNSLTSEDSAVYFCQRQLGQGYWGQGTTLTVSS

SEQ ID NO: 24 - protein, 113 aa, Artificial Sequence
  Description of Artificial Sequence: Synthetic polypeptide
DVVMTQTPLSLPVSLGDQASISCRSSQSLVHSYGNTYLHWYLQKPGQSPKLLIYKVSNRFSGVPDRFSGSGSGTDFTLKISRVEAEDLGVYFCSQNTHVPYTFGGGTKLEIKR

SEQ ID NO: 25 - protein, 115 aa, Artificial Sequence
  Description of Artificial Sequence: Synthetic polypeptide
QVQLQQSDAELGKPGASVKISCKASGYTFSDHAIHWVKQKPEQGLEWIGYISPGNDDIKYNEKFKGKATLTADKSSSTAYMQLNSLTSEDSAVYFCERSMIGVYWGQGTLVTVSA

SEQ ID NO: 26 - protein, 112 aa, Artificial Sequence
  Description of Artificial Sequence: Synthetic polypeptide
DVVMTQTPLSLTVSLGDQASISCRFSQSLVQSNGNTYLQWYLQKPGQSPKLLIYKVSNRFCGVPDRFSGSGSGTDFTLKISRVEAEDLGVYFCSQSTHAPLTFGAGTKLELK

SEQ ID NO: 27 - protein, 114 aa, Artificial Sequence
  Description of Artificial Sequence: Synthetic polypeptide
QVQLQQSDAELVKPGASVKISCKTSGYTFTDHAIHWVKQKPEQGLEWIGYISPGNGDIKYNEKFKGKATLTADKSSSTAYMQLSSLTPEDSAVYFCKISYYGIWGQGTTLTVSS

SEQ ID NO: 28 - protein, 107 aa, Artificial Sequence
  Description of Artificial Sequence: Synthetic polypeptide
DIQMTQSPASLSVSVGESVTITCRLSEDIYSNLAWFQQRPGKSPQLLVYKATNLADGVPSRFSGSGSGTQYSLKINSLQSEDFGTYYCQHFWGTPFTFGSGTKVEIK

SEQ ID NO: 29 - protein, 114 aa, Artificial Sequence
  Description of Artificial Sequence: Synthetic polypeptide
QVQLQQSDAELVKPGASVKISCKASGYTFTDHAIHWVKQKPEQGLEWIGYFSPGNDDIKYNEKFKVKATLTADKSSSTAYMQLTSLTSEDSAVYFCKRSYYGDWGQGTTLTVSS

SEQ ID NO: 30 - protein, 107 aa, Artificial Sequence
  Description of Artificial Sequence: Synthetic polypeptide
DIQMTQSPASLSVSVGETVTITCRASENIYSHLAWYQQKQGKSPQLLVYGATNLADGVPSRFSGSGSGTQFSLKIHSLQSEDFGSYYCQHFWGAPFTFGSGTKLEIK

SEQ ID NO: 31 - protein, 115 aa, Artificial Sequence
  Description of Artificial Sequence: Synthetic polypeptide
QIQLQQSDAELVKPGTSVKMSCKASGYTFTDHAIHWVKQKPEQGLEWIGYFSPGNDDIKYNVKFKGKATLTADKSSSTAYMQLNSLTSEDSAVYFCSVGYALDYWGLGTTLTVSS

SEQ ID NO: 32 - protein, 108 aa, Artificial Sequence
  Description of Artificial Sequence: Synthetic polypeptide
NIVMTQSPKSMSMSVGERVTLTCKASENVVTYVSWYQQKPEQSPKLLIYGASNRYTGVPDRFTGSGSATDFTLTISSVQAEDLADYHCGQGYSYPYTFGGGTKLEIKR

SEQ ID NO: 33 - protein, 115 aa, Artificial Sequence
  Description of Artificial Sequence: Synthetic polypeptide
QVQLQQSDAELVKPGTTVKISCKASGYTFTDHAIHWVKEKPEQGLEWIGYISPGNDDIKYSEKFKGKATLTADKSSSTAYMQLNSLTSDDSAVYFCKRSLSTPYWGQGTLVTVSA

SEQ ID NO: 34 - protein, 114 aa, Artificial Sequence
  Description of Artificial Sequence: Synthetic polypeptide
DIVMTQSPSSLTVTAGEKVTMSCRSSQSLLNSGNQKNYLTWYQQKPGQPPKLLIYWASTRESGVPDRFTGSGSGTDFTLTISSVQAEDLAVYYCQNDYSYPYTFGGGTKLEIKR

SEQ ID NO: 35 - protein, 114 aa, Artificial Sequence
  Description of Artificial Sequence: Synthetic polypeptide
QVQLQQSDAELVKPGASVKISCKASGYTFTDHAIHWVMQMPEQGLEWIGYISPGNGDVKYSERFKGRATLTADKSSSSAYMQLNSLTSEDSAVYFCKRSLSTPYWGQGTLVTVS

SEQ ID NO: 36 - protein, 114 aa, Artificial Sequence
  Description of Artificial Sequence: Synthetic polypeptide
DIVMTQSPSSLTVTAGERVTMSCKSSQSLLNSGNQKSYLTWYQQKPGQPPKLLISWASTRDSGVPDRFTGSGSGTDFTLTISSVQAEDLAVYYCQSDYSYPYTFGGGTKLEIKR

SEQ ID NO: 37 - protein, 115 aa, Artificial Sequence
  Description of Artificial Sequence: Synthetic polypeptide
  MOD_RES (9)..(9): Any amino acid or not present
  MOD_RES (111)..(111): Any amino acid or not present
QVQLQQSDXELVKPGASVKISCKASGYTFTDHAIHWVKQKPEQGLEWIGYFSPGNDDIKYNEKFRGKATLTADKSSSTAYMQLNSLSSDDSAVYFCKRSLSTPYWGQGTLXTVSA

SEQ ID NO: 38 - protein, 114 aa, Artificial Sequence
  Description of Artificial Sequence: Synthetic polypeptide
DIVMTQSPSSLTVTAGEKVTMSCKSSQSLLNRGNHKNYLTWYRQKPGLPPKLLIYWASTRESGVPDRFTGSGSGTDFALTISSVQAEDLAVYYCQNDYTYPYTFGGGTKLEIKR

SEQ ID NO: 39 - protein, 115 aa, Artificial Sequence
  Description of Artificial Sequence: Synthetic polypeptide
QVQLQQSDAELVKPGASMKISCKASGYTFTDHAIHWVKQKPEQGLEWIGYISPGNGDIKYNEKFKVKATLTADKSSSTAYMQLNSLTSEDSAVYFCKRSITTPYWGQGTLVTVSA

SEQ ID NO: 40 - protein, 114 aa, Artificial Sequence
  Description of Artificial Sequence: Synthetic polypeptide
DIVMTQSPSSLTVTAGEKVTMSCKSSQSLLNSGKTKNYLTWYQQKPGQPPKLLIYWASTRESGVPDRFTGSGSGTDFTLTISSVQAEDLAVYYCKNDYSYPYTFGGGTKLEIKR

SEQ ID NO: 41 - protein, 115 aa, Artificial Sequence
  Description of Artificial Sequence: Synthetic polypeptide
QVQLQQSDAELVKPGASVKISCKTSGYTFTDHAIHWVKQKPEQGLEWIGYISPGNDDIKYTEKFKGKVTLTADKSSSTAYMQLNSLTSEDSAVYFCKRSITTPYWGQGTLVTVSA

SEQ ID NO: 42 - protein, 115 aa, Artificial Sequence
  Description of Artificial Sequence: Synthetic polypeptide
QVQLQQSDAELVKPGASVKISCKASGYTFTDHAIHWVKQKPEQGLEWIGYISPGNGDIKYDEKFKGKATLTADKSSSTAYMQLNSLTSEDSAVYFCKRSITTSYWGQGTLVTVSA

SEQ ID NO: 43 - protein, 115 aa, Artificial Sequence
  Description of Artificial Sequence: Synthetic polypeptide
QVQLQQSDAELVKPGASVKISCKASGYTFTDHAIHWVKQKPEQGLEWIGYISPGNDDIKYNEKFKGKATLTADKSSSTAYMQLNSLTSEDSAVFFCKRSITTSYWGQGTLVTVSA

SEQ ID NO: 44 - protein, 115 aa, Artificial Sequence
  Description of Artificial Sequence: Synthetic polypeptide
QVQLQQSDAELVKPGASVKISCKASGYIFTDHAIHWVKQKPEQGLEWIGYISPGNGDIKYNEKFKGKATLTADKSSSTAYMHLNSLTSEDSAVYFCKRSITTSYWGQGTLVTVSA

SEQ ID NO: 45 - protein, 108 aa, Artificial Sequence
  Description of Artificial Sequence: Synthetic polypeptide
DIQMNQSPSSLSASLGDTITITCHASQHINFWLSWYQQKPGNIPKLLIYKASNLHTGVPSRFSGSGSGTGFTLTISSLLPEDVATYYCQQDQSYPYMFGGGTKLEIKR

SEQ ID NO: 46 - protein, 115 aa, Artificial Sequence
  Description of Artificial Sequence: Synthetic polypeptide
QVQLQQSDAELVKPGASVKISCKASGYTFTDHAIHWVKQKPEQGLEWIGYISPGNDDIKYNEKFKGKATLTADKSSSTAYMLLNSLTSEDSAVYFCKRSITTSYWGQGTLVTVSA

SEQ ID NO: 47 - protein, 115 aa, Artificial Sequence
  Description of Artificial Sequence: Synthetic polypeptide
QVQLQQSDAELVKPGASVKISCKASGYTFTDHAIHWVKQKPEQGLEWIGYISPGNGDIKYNEKFKGKATLTADTSSTTAYMQLNSLTSEDSAMYFCKRSITTSYWGQGTLVTVSA

SEQ ID NO: 48 - protein, 115 aa, Artificial Sequence
  Description of Artificial Sequence: Synthetic polypeptide
QVQLQQSDAELVKPGASVKISCKASGYIFTDHAIHWVKQKPEQGLEWIGYISPGNGDIKYIEKFRGKATLTADKSSSTAYMQLNSLTSEDSAVYFCKRSLSTPYWGQGTLVTVSA

SEQ ID NO: 49 - protein, 110 aa, Artificial Sequence
  Description of Artificial Sequence: Synthetic polypeptide
NILMTQSPKSMSMSVGERVTLTCKASENVVNYVSWYQQKPEQSPKLLIFGASNRYSGVPDRFTGSGSATDFTLTISSVQAEDLADYHCGSKWITSYPYTFGGGTKLEIKR

SEQ ID NO: 50 - protein, 109 aa, Artificial Sequence
  Description of Artificial Sequence: Synthetic polypeptide
NILMTQSPKSMSMSVGERVTLTCKASENVVNYVSWYQQKPEQSPKLLIYGASNRYSGVPDRFTGSGSATDFTLTISSVQAEDLADYHCGARVTSYPYTFGGGTKLEIKR

SEQ ID NO: 51 - protein, 115 aa, Artificial Sequence
  Description of Artificial Sequence: Synthetic polypeptide
QVQLQQSDAELVKPGTSVKISCRASGYTFTDHAIHWVKQKPEQGLEWIGYISPGNGDIKYNEKFKGKATLTADKSSSTAYMQLNSLTSDDSAVYFCKRSITTPYWGQGTTLTVSS

SEQ ID NO: 52 - protein, 105 aa, Artificial Sequence
  Description of Artificial Sequence: Synthetic polypeptide
SFVMTQTPKFLLVSAGDRVTITCKASQSVNNNVAWYQQKPGQSPKQLIYYASNRYTGVPDRFTGSGYGTDFTFTIYTVQAEDLAVYFCQQGYSSPWTFGGGTKLK

SEQ ID NO: 53 - protein, 116 aa, Artificial Sequence
  Description of Artificial Sequence: Synthetic polypeptide
QVQLQQSDAELVKPGASVKISCKASGYTFTDHAIHWVKQKPEQGLDWIGYISPGNGDIKYNEKFKDKVTLTADKSSSTACMHLNSLTSEDSAVYFCKRSLLALDYWGQGTTLTVSS

SEQ ID NO: 54 - protein, 107 aa, Artificial Sequence
  Description of Artificial Sequence: Synthetic polypeptide
DIVMTQSHKFMSTSVGDRVSITCKASQDVGTNIAWYQQKPGRSPKVLIYSASTRHTGVPDRFTGSGSGTDFTLTISNVQSEDLTDYFCQQYSSFPLTFGVGTKLELK

SEQ ID NO: 55 - protein, 10 aa, Artificial Sequence
  Description of Artificial Sequence: Synthetic peptide
GFSLSTSNMG

SEQ ID NO: 56 - protein, 10 aa, Artificial Sequence
  Description of Artificial Sequence: Synthetic peptide
GFSLSTFGMG

SEQ ID NO: 57 - protein, 8 aa, Artificial Sequence
  Description of Artificial Sequence: Synthetic peptide
GFSLTSYG

SEQ ID NO: 58 - protein, 8 aa, Artificial Sequence
  Description of Artificial Sequence: Synthetic peptide
GFSLISYG

SEQ ID NO: 59 - protein, 7 aa, Artificial Sequence
  Description of Artificial Sequence: Synthetic peptide
IWWHDDK

SEQ ID NO: 60 - protein, 7 aa, Artificial Sequence
  Description of Artificial Sequence: Synthetic peptide
IWWDDDK

SEQ ID NO: 61 - protein, 7 aa, Artificial Sequence
  Description of Artificial Sequence: Synthetic peptide
IWGDGST

SEQ ID NO: 62 - protein, 13 aa, Artificial Sequence
  Description of Artificial Sequence: Synthetic peptide
AQVPFYYGTSFDV

SEQ ID NO: 63 - protein, 13 aa, Artificial Sequence
  Description of Artificial Sequence: Synthetic peptide
ARIAYYYGSERDY

SEQ ID NO: 64 - protein, 6 aa, Artificial Sequence
  Description of Artificial Sequence: Synthetic peptide
ARAFVY

SEQ ID NO: 65 - protein, 6 aa, Artificial Sequence
  Description of Artificial Sequence: Synthetic peptide
TKGFTY

SEQ ID NO: 66 - protein, 6 aa, Artificial Sequence
  Description of Artificial Sequence: Synthetic peptide
TKGFAY

SEQ ID NO: 67 - protein, 6 aa, Artificial Sequence
  Description of Artificial Sequence: Synthetic peptide
TKGFVY

SEQ ID NO: 68 - protein, 8 aa, Artificial Sequence
  Description of Artificial Sequence: Synthetic peptide
AKGGYFDY

SEQ ID NO: 69 - protein, 5 aa, Artificial Sequence
  Description of Artificial Sequence: Synthetic peptide
SSISY

SEQ ID NO: 70 - protein, 5 aa, Artificial Sequence
  Description of Artificial Sequence: Synthetic peptide
SSVSY

SEQ ID NO: 71 - protein, 6 aa, Artificial Sequence
  Description of Artificial Sequence: Synthetic peptide
QSISDY

SEQ ID NO: 72 - protein, 5 aa, Artificial Sequence
  Description of Artificial Sequence: Synthetic peptide
SSITY

SEQ ID NO: 73 - protein, 3 aa, Artificial Sequence
  Description of Artificial Sequence: Synthetic peptide
DTS

SEQ ID NO: 74 - protein, 3 aa, Artificial Sequence
  Description of Artificial Sequence: Synthetic peptide
STS

SEQ ID NO: 75 - protein, 3 aa, Artificial Sequence
  Description of Artificial Sequence: Synthetic peptide
YAS

SEQ ID NO: 76 - protein, 7 aa, Artificial Sequence
  Description of Artificial Sequence: Synthetic peptide
HQRSSYT

SEQ ID NO: 77 - protein, 11 aa, Artificial Sequence
  Description of Artificial Sequence: Synthetic peptide
QQWSSNPPMLT

SEQ ID NO: 78 - protein, 9 aa, Artificial Sequence
  Description of Artificial Sequence: Synthetic peptide
QQWSSNLLT

SEQ ID NO: 79 - protein, 9 aa, Artificial Sequence
  Description of Artificial Sequence: Synthetic peptide
QQRSSYPWT

SEQ ID NO: 80 - protein, 9 aa, Artificial Sequence
  Description of Artificial Sequence: Synthetic peptide
QNGHSFPLT

SEQ ID NO: 81 - protein, 12 aa, Artificial Sequence
  Description of Artificial Sequence: Synthetic peptide
GYTFTDHAIHWV

SEQ ID NO: 82 - protein, 12 aa, Artificial Sequence
  Description of Artificial Sequence: Synthetic peptide
GYTFSDHAIHWV

SEQ ID NO: 83 - protein, 12 aa, Artificial Sequence
  Description of Artificial Sequence: Synthetic peptide
GYIFTDHAIHWV

SEQ ID NO: 84 - protein, 10 aa, Artificial Sequence
  Description of Artificial Sequence: Synthetic peptide
FSPGNDDIKY

SEQ ID NO: 85 - protein, 10 aa, Artificial Sequence
  Description of Artificial Sequence: Synthetic peptide
ISPGNGDIKY

SEQ ID NO: 86 - protein, 10 aa, Artificial Sequence
  Description of Artificial Sequence: Synthetic peptide
LSPGNDDIKY

SEQ ID NO: 87 - protein, 10 aa, Artificial Sequence
  Description of Artificial Sequence: Synthetic peptide
VSPGNGDIKY

SEQ ID NO: 88 - protein, 10 aa, Artificial Sequence
  Description of Artificial Sequence: Synthetic peptide
ISPGNGDVKY

SEQ ID NO: 89 - protein, 10 aa, Artificial Sequence
  Description of Artificial Sequence: Synthetic peptide
ISPGNDDIKY

SEQ ID NO: 90 - protein, 8 aa, Artificial Sequence
  Description of Artificial Sequence: Synthetic peptide
SVGYALDY

SEQ ID NO: 91 - protein, 7 aa, Artificial Sequence
  Description of Artificial Sequence: Synthetic peptide
KISYYGI

SEQ ID NO: 92 - protein, 7 aa, Artificial Sequence
  Description of Artificial Sequence: Synthetic peptide
KRSYYGD

SEQ ID NO: 93 - protein, 8 aa, Artificial Sequence
  Description of Artificial Sequence: Synthetic peptide
KRSIGGDH

SEQ ID NO: 94 - protein, 8 aa, Artificial Sequence
  Description of Artificial Sequence: Synthetic peptide
QRQLGQGY

SEQ ID NO: 95 - protein, 8 aa, Artificial Sequence
  Description of Artificial Sequence: Synthetic peptide
KRSLIGDY

SEQ ID NO: 96 - protein, 8 aa, Artificial Sequence
  Description of Artificial Sequence: Synthetic peptide
KRSLSTPY

SEQ ID NO: 97 - protein, 8 aa, Artificial Sequence
  Description of Artificial Sequence: Synthetic peptide
KRSITTPY

SEQ ID NO: 98 - protein, 8 aa, Artificial Sequence
  Description of Artificial Sequence: Synthetic peptide
ERSMIGVY

SEQ ID NO: 99 - protein, 8 aa, Artificial Sequence
  Description of Artificial Sequence: Synthetic peptide
KRSITTSY

SEQ ID NO: 100 - protein, 6 aa, Artificial Sequence
  Description of Artificial Sequence: Synthetic peptide
ENVVTY

SEQ ID NO: 101 - protein, 6 aa, Artificial Sequence
  Description of Artificial Sequence: Synthetic peptide
EDIYSN

SEQ ID NO: 102 - protein, 6 aa, Artificial Sequence
  Description of Artificial Sequence: Synthetic peptide
ENIYSH

SEQ ID NO: 103 - protein, 6 aa, Artificial Sequence
  Description of Artificial Sequence: Synthetic peptide
QNINVW

SEQ ID NO: 104 - protein, 11 aa, Artificial Sequence
  Description of Artificial Sequence: Synthetic peptide
QSLVHSYGNTY

SEQ ID NO: 105 - protein, 6 aa, Artificial Sequence
  Description of Artificial Sequence: Synthetic peptide
QNVGTA

SEQ ID NO: 106 - protein, 12 aa, Artificial Sequence
  Description of Artificial Sequence: Synthetic peptide
QSLLNSGNQKSY

SEQ ID NO: 107 - protein, 6 aa, Artificial Sequence
  Description of Artificial Sequence: Synthetic peptide
QSVNNN

SEQ ID NO: 108 - protein, 12 aa, Artificial Sequence
  Description of Artificial Sequence: Synthetic peptide
QSLLNRGNHKNY

SEQ ID NO: 109 - protein, 11 aa, Artificial Sequence
  Description of Artificial Sequence: Synthetic peptide
QSLVQSNGNTY

SEQ ID NO: 110 - protein, 6 aa, Artificial Sequence
  Description of Artificial Sequence: Synthetic peptide
ENVVNY

SEQ ID NO: 111 - protein, 12 aa, Artificial Sequence
  Description of Artificial Sequence: Synthetic peptide
QSLLNSGKTKNY

SEQ ID NO: 112 - protein, 6 aa, Artificial Sequence
  Description of Artificial Sequence: Synthetic peptide
QHINFW

SEQ ID NO: 113 - protein, 6 aa, Artificial Sequence
  Description of Artificial Sequence: Synthetic peptide
ENVVIY

SEQ ID NO: 114 - protein, 12 aa, Artificial Sequence
  Description of Artificial Sequence: Synthetic peptide
QSLLNSGNQKNY

SEQ ID NO: 115 - protein, 7 aa, Artificial Sequence
  Description of Artificial Sequence: Synthetic peptide
GASNRYT

SEQ ID NO: 116 - protein, 7 aa, Artificial Sequence
  Description of Artificial Sequence: Synthetic peptide
KATNLAD

SEQ ID NO: 117 - protein, 7 aa, Artificial Sequence
  Description of Artificial Sequence: Synthetic peptide
GATNLAD

SEQ ID NO: 118 - protein, 7 aa, Artificial Sequence
  Description of Artificial Sequence: Synthetic peptide
KASNLHT

SEQ ID NO: 119 - protein, 7 aa, Artificial Sequence
  Description of Artificial Sequence: Synthetic peptide
KVSNRFS

SEQ ID NO: 120 - protein, 7 aa, Artificial Sequence
  Description of Artificial Sequence: Synthetic peptide
SASNRYT

SEQ ID NO: 121 - protein, 7 aa, Artificial Sequence
  Description of Artificial Sequence: Synthetic peptide
WASTRDS

SEQ ID NO: 122 - protein, 7 aa, Artificial Sequence
  Description of Artificial Sequence: Synthetic peptide
YASNRYT

SEQ ID NO: 123 - protein, 7 aa, Artificial Sequence
  Description of Artificial Sequence: Synthetic peptide
WASTRES

SEQ ID NO: 124 - protein, 7 aa, Artificial Sequence
  Description of Artificial Sequence: Synthetic peptide
KVSNRFC

SEQ ID NO: 125 - protein, 7 aa, Artificial Sequence
  Description of Artificial Sequence: Synthetic peptide
GASNRYS

SEQ ID NO: 126 - protein, 7 aa, Artificial Sequence
  Description of Artificial Sequence: Synthetic peptide
KVSNLHT

SEQ ID NO: 127 - protein, 9 aa, Artificial Sequence
  Description of Artificial Sequence: Synthetic peptide
GQGYSYPYT

SEQ ID NO: 128 - protein, 9 aa, Artificial Sequence
  Description of Artificial Sequence: Synthetic peptide
QHFWGTPFT

SEQ ID NO: 129 - protein, 9 aa, Artificial Sequence
  Description of Artificial Sequence: Synthetic peptide
QHFWGAPFT

SEQ ID NO: 130 - protein, 9 aa, Artificial Sequence
  Description of Artificial Sequence: Synthetic peptide
QQGQSYPFT

SEQ ID NO: 131 - protein, 9 aa, Artificial Sequence
  Description of Artificial Sequence: Synthetic peptide
SQNTHVPYT

SEQ ID NO: 132 - protein, 9 aa, Artificial Sequence
  Description of Artificial Sequence: Synthetic peptide
QQYSSYRLT

SEQ ID NO: 133 - protein, 9 aa, Artificial Sequence
  Description of Artificial Sequence: Synthetic peptide
QSDYSYPYT

SEQ ID NO: 134 - protein, 9 aa, Artificial Sequence
  Description of Artificial Sequence: Synthetic peptide
QQGYSSPWT

SEQ ID NO: 135 - protein, 9 aa, Artificial Sequence
  Description of Artificial Sequence: Synthetic peptide
QNDYTYPYT

SEQ ID NO: 136 - protein, 9 aa, Artificial Sequence
  Description of Artificial Sequence: Synthetic peptide
SQSTHAPLT

SEQ ID NO: 137 - protein, 11 aa, Artificial Sequence
  Description of Artificial Sequence: Synthetic peptide
GSKWITSYPYT

SEQ ID NO: 138 - protein, 10 aa, Artificial Sequence
  Description of Artificial Sequence: Synthetic peptide
GARVTSYPYT

SEQ ID NO: 139 - protein, 9 aa, Artificial Sequence
  Description of Artificial Sequence: Synthetic peptide
QQDQSYPYT

SEQ ID NO: 140 - protein, 9 aa, Artificial Sequence
  Description of Artificial Sequence: Synthetic peptide
KNDYSYPYT

SEQ ID NO: 141 - protein, 9 aa, Artificial Sequence
  Description of Artificial Sequence: Synthetic peptide
QQDQSYPYM

SEQ ID NO: 142 - protein, 9 aa, Artificial Sequence
  Description of Artificial Sequence: Synthetic peptide
QNDYSYPYT

SEQ ID NO: 143 - protein, 10 aa, Artificial Sequence
  Description of Artificial Sequence: Synthetic peptide
GYTFTDHAIH

SEQ ID NO: 144 - protein, 10 aa, Artificial Sequence
  Description of Artificial Sequence: Synthetic peptide
GYIFTDHAIH

SEQ ID NO: 145 - protein, 17 aa, Artificial Sequence
  Description of Artificial Sequence: Synthetic peptide
YISPGNGDIKYNEKFKG

SEQ ID NO: 146 - protein, 17 aa, Artificial Sequence
  Description of Artificial Sequence: Synthetic peptide
YFSPGNDDIKYNEKFRG

SEQ ID NO: 147 - protein, 17 aa, Artificial Sequence
  Description of Artificial Sequence: Synthetic peptide
YFSPGNDDIKYNEKFKV

SEQ ID NO: 148 - protein, 17 aa, Artificial Sequence
  Description of Artificial Sequence: Synthetic peptide
YISPGNGDIKYNEKFKV

SEQ ID NO: 149 - protein, 17 aa, Artificial Sequence
  Description of Artificial Sequence: Synthetic peptide
YISPGNGDIKYNEKFKD

SEQ ID NO: 150 - protein, 17 aa, Artificial Sequence
  Description of Artificial Sequence: Synthetic peptide
YFSPGNDDFKYNEKFKG

SEQ ID NO: 151 - protein, 17 aa, Artificial Sequence
  Description of Artificial Sequence: Synthetic peptide
YISPGNDDIKYNEKFKG

SEQ ID NO: 152 - protein, 6 aa, Artificial Sequence
  Description of Artificial Sequence: Synthetic peptide
SITTSY

SEQ ID NO: 153 - protein, 6 aa, Artificial Sequence
  Description of Artificial Sequence: Synthetic peptide
SLSTPY

SEQ ID NO: 154 - protein, 5 aa, Artificial Sequence
  Description of Artificial Sequence: Synthetic peptide
SYYGD

SEQ ID NO: 155 - protein, 6 aa, Artificial Sequence
  Description of Artificial Sequence: Synthetic peptide
SITTPY

SEQ ID NO: 156 - protein, 7 aa, Artificial Sequence
  Description of Artificial Sequence: Synthetic peptide
SLLALDY

SEQ ID NO: 157 - protein, 6 aa, Artificial Sequence
  Description of Artificial Sequence: Synthetic peptide
SLNMAY

SEQ ID NO: 158 - protein, 5 aa, Artificial Sequence
  Description of Artificial Sequence: Synthetic peptide
SYYGH

SEQ ID NO: 159 - protein, 11 aa, Artificial Sequence
  Description of Artificial Sequence: Synthetic peptide
KASENVVTYVS

SEQ ID NO: 160 - protein, 11 aa, Artificial Sequence
  Description of Artificial Sequence: Synthetic peptide
HASQHINFWLS

SEQ ID NO: 161 - protein, 17 aa, Artificial Sequence
  Description of Artificial Sequence: Synthetic peptide
KSSQSLLNRGNHKNYLT

SEQ ID NO: 162 - protein, 11 aa, Artificial Sequence
  Description of Artificial Sequence: Synthetic peptide
RASENIYSHLA

SEQ ID NO: 163 - protein, 17 aa, Artificial Sequence
  Description of Artificial Sequence: Synthetic peptide
KSSQSLLNSGKTKNYLT

SEQ ID NO: 164 - protein, 11 aa, Artificial Sequence
  Description of Artificial Sequence: Synthetic peptide
KASQSVNNNVA

SEQ ID NO: 165 - protein, 11 aa, Artificial Sequence
  Description of Artificial Sequence: Synthetic peptide
KASQDVGTNIA

SEQ ID NO: 166 - protein, 17 aa, Artificial Sequence
  Description of Artificial Sequence: Synthetic peptide
KSSQSLLYSGNQKNYLA

SEQ ID NO: 167 - protein, 11 aa, Artificial Sequence
  Description of Artificial Sequence: Synthetic peptide
RASENIYSNLA

SEQ ID NO: 168 - protein, 7 aa, Artificial Sequence
  Description of Artificial Sequence: Synthetic peptide
SASTRHT

SEQ ID NO: 169 - protein, 7 aa, Artificial Sequence
  Description of Artificial Sequence: Synthetic peptide
WASARES

SEQ ID NO: 170 - protein, 7 aa, Artificial Sequence
  Description of Artificial Sequence: Synthetic peptide
AATNLAD

SEQ ID NO: 171 - protein, 9 aa, Artificial Sequence
  Description of Artificial Sequence: Synthetic peptide
QQYSSFPLT

SEQ ID NO: 172 - protein, 9 aa, Artificial Sequence
  Description of Artificial Sequence: Synthetic peptide
QQYYSYPLT

SEQ ID NO: 173 - protein, 9 aa, Artificial Sequence
  Description of Artificial Sequence: Synthetic peptide
QHFWGTPYT

SEQ ID NO: 174 - DNA, 363 bp, Artificial Sequence
  Description of Artificial Sequence: Synthetic polynucleotide
caggttactctgaaagagtctggccctgggatattgcagccctcccagaccctcagtctgacttgttctttctctgggttttcactgagcacttctaatatgggtataggctggattcgtcagccttcagggaagggtctagagtggctggcacacatttggtggcatgatgataagtactataacccatccctgaagagccggctcacaatctccaaggatatctccaacaaccaggtattcctcaagatcaccagtgtggacactgcagatactgccacgtactactgtgctcaagtcccgttttactacggaacctcgttcgatgtctggggcacagggaccacggtcaccgtctcctca

SEQ ID NO: 175 - DNA, 322 bp, Artificial Sequence
  Description of Artificial Sequence: Synthetic polynucleotide
gacattgtgatgactcagtctccagccaccctgtctgtgactccaggagatagagtctctctttcctgcagggccagccagagtattagcgactacttacactggtatcaacaaaaatcacatgagtctccaaggcttctcatcaaatatgcttcccaatccatctctgggatcccctccaggttcagtggcagtggatcagggtcagatttcactctcagtatcaacagtgtggaacctgaagatgttggagtgtattactgtcaaaatggtcacagctttcctctcacgttcggtgctgggaccaagctggagctgaaac

SEQ ID NO: 176 - DNA, 314 bp, Artificial Sequence
  Description of Artificial Sequence: Synthetic polynucleotide
caaattgttctcacccagtctccagcaatcatgtctgcatctccaggggagacggtcaccatgacctgcagtgccagctcaagtataacttacatgcactggtaccagcagaagccaggcacctcccccaaaagatggatttatgacacatccaaactggcttctggagtccctgctcgcttcagtggcagtgggtctgggacctcttattctctcacaatcagcagcatggaggctgaagatgctgccacttattactgccatcagcggagtagttacacgttcggaggggggaccaagctggaaataaaacg

SEQ ID NO: 177 - DNA, 363 bp, Artificial Sequence
  Description of Artificial Sequence: Synthetic polynucleotide
caggttactctgaaagagtctggccctgggatattgcagccctcccagaccctcagtctgacttgttctttctctgggttttcactgagcacttttggtatgggtgtaggctggattcgtcagccttcagggaagggtctggagtggctggcacacatttggtgggatgatgataagtactataacccagccctgaagagtcggctcacaatctccaaggatacctccaaaaaccaggtattcctcaagatcgccaatgtggacactgcagatactgccacatactactgtgctcgaatagcctattactacggtagcgagagggactactggggccaaggcaccactctcacagtctcctca

SEQ ID NO: 178 - DNA, 314 bp, Artificial Sequence
  Description of Artificial Sequence: Synthetic polynucleotide
caaattgttctcacccagtctccagcaatcatgtctgcatctccaggggagaaggtcaccatgacctgcagtgccagctcaagtataagttacatgcactggtaccaccagaagccaggcacctcccccaaaagatggatttatgacacatccaaactggcttctggagtccctgctcgcttcagtggcagtgggtctgggacctcttattctctcacaatcagcagcatggaggctgaagatgctgccacttattactgccatcagcggagtagttacacgttcggaggggggaccaagctggaaataaaacg

SEQ ID NO: 179 - DNA, 1047 bp, Artificial Sequence
  Description of Artificial Sequence: Synthetic polynucleotide
atggacaggcttacttcctcattcttgctactgattgtccctgcatatgtcctgtcccaggttactctgaaagagtctggccctgggatattgcagccctcccagaccctcagtctgacttgttctttctctgggttttcactgagcacttctaatatgggtataggctggattcgtcagccttcagggaagggtctagagtggctggcacacatttggtggcatgatgataagtactataacccatccctgaagagccggctcacaatctccaaggatatctccaacaaccaggtattcctcaagatcaccagtgtggacactgcagatactgccacgtactactgtgctcaagtcccgttttactacggaacctcgttcgatgtctggggcacagggaccacggtcaccgtctcctcagccaaaacgacacccccatctgtctatccgctcgcccctggatctgctgcccaaactaactccatggtgaccctgggatgcctggtcaagggctatttccctgagccagtgacagtgacctggaactctggatccctgtccagcggtgtgcacaccttcccagctgtcctgcagtctgacctctacactctgagcagctcagtgactgtcccctccagcacctggcccagcgagaccgtcacctgcaacgttgcccacccggccagcagcaccaaggtggacaagacaattgtgcccagggattgtggttgtaagccttgcatatgtacagtcccagaagtatcatctgtcttcatcttccccccaaagcccaaggatgtgctcaccattactctgactcctaaggtcacgtgtgttgtggtagacatcagccaggatgatcccgaggtcagttcagctgtttgtagatgatgtggaagtgcacacagctcaaaacaaccccccgagaggacatttcacaacatttccgctcatcagtgaatttcccatctgcacaagactgcttaatggcaagagttaaatgcaggtcaaagggcagtttcctgccccatcaaaaacttttcaaaa

SEQ ID NO: 180 - DNA, 702 bp, Artificial Sequence
  Description of Artificial Sequence: Synthetic polynucleotide
atggattttcaagtgcagattttcagcttcctgctaatcagtgcctcagtcatactgtccagaggacaaattgttctcacccagtctccagcaatcatgtctgcatctccaggggagacggtcaccatgacctgcagtgccagctcaagtataacttacatgcactggtaccagcagaagccaggcacctcccccaaaagatggatttatgacacatccaaactggcttctggagtccctgctcgcttcagtggcagtgggtctgggacctcttattctctcacaatcagcagcatggaggctgaagatgctgccacttattactgccatcagcggagtagttacacgttcggaggggggaccaagctggaaataaaacgggctgatgctgcaccaactgtatccatcttcccaccatccagtgagcagttaacatctggaggtgcctcagtcgtgtgcttcttgaacaacttctaccccaaagacatcaatgtcaagtggaagattgatggcagtgaacgacaaaatggcgtcctgaacagttggactgatcaggacagcaaagacagcacctacagcatgagcagcaccctcacgttgaccaaggacgagtatgaacgacataacagctatacctgtgaggccactcacaagacatcaacttcacccattgtcaagagcttcaacaggaatgagtgttag

SEQ ID NO: 181 - DNA, 1252 bp, Artificial Sequence
  Description of Artificial Sequence: Synthetic polynucleotide
  modified_base (919)..(919): a, c, g, t or not present
  modified_base (984)..(984): a, c, g, t or not present
  modified_base (999)..(999): a, c, g, t or not present
  modified_base (1011)..(1011): a, c, g, t or not present
  modified_base (1057)..(1057): a, c, g, t or not present
  modified_base (1100)..(1100): a, c, g, t or not present
  modified_base (1201)..(1201): a, c, g, t or not present
atggacaggcttacttcctcattcctgttactgattgtccctgcatatgtcctgtcccaggttactctgaaagagtctggccctgggatattgcagccctcccagaccctcagtctgacttgttctttctctgggttttcactgagcacttttggtatgggtgtaggctggattcgtcagccttcagggaagggtctggagtggctggcacacatttggtgggatgatgataagtactataacccagccctgaagagtcggctcacaatctccaaggatacctccaaaaaccaggtattcctcaagatcgccaatgtggacactgcagatactgccacatactactgtgctcgaatagcctattactacggtagcgagagggactactggggccaaggcaccactctcacagtctcctcagccaaaacgacacccccatctgtctatccgctcgcccctggatctgctgcccaaactaactccatggtgaccctgggatgcctggtcaagggctatttccctgagccagtgacagtgacctggaactctggatccctgtccagcggtgtgcacaccttcccagctgtcctgcagtctgacctctacactctgagcagctcagtgactgtcccctccagcacctggcccagcgagaccgtcacctgcaacgttgcccacccggccagcagcaccaaggtggacaagaaaattgtgcccagggattgtggttgtaagccttgcatatgtacagtcccagaagtatcatctgtcttcatcttccccccaaagcccaaggatgtgctcaccattactctgactcctaaggtcacgtgtgttgtggtagacatcagcaaggatgatcccgaggtccagttcagctggtttgtagatgatgtggaagtgcacacagctcagacgncaccccggggagagcagtttcacagcactttccgctcagtcagtgaacttcccatcatgcaccangactgggctcatggncaggagttcaantgcaggtcacagtgcagctttcctgccccatcgagaaacatctccnaaacaaggcgacgaaagctcacagggtacacattccactcccnagagcaatgccagataagtcatctgactgctgatacaactcttctgaaaatactgtgaatgcatggatgccaccacgaaaatcaaacctcgcccttggacnatggcttattttaccagctagtcaaaacctggggggaatttcccgtctgtt

SEQ ID NO: 182 - DNA, 705 bp, Artificial Sequence
  Description of Artificial Sequence: Synthetic polynucleotide
atggttttcacacctcagatacttggacttatgcttttttggatttcagcctccagatgtgacattgtgatgactcagtctccagccaccctgtctgtgactccaggagatagagtctctctttcctgcagggccagccagagtattagcgactacttacactggtatcaacaaaaatcacatgagtctccaaggcttctcatcaaatatgcttcccaatccatctctgggatcccctccaggttcagtggcagtggatcagggtcagatttcactctcagtatcaacagtgtggaacctgaagatgttggagtgtattactgtcaaaatggtcacagctttcctctcacgttcggtgctgggaccaagctggaaataaaacgggctgatgctgcaccaactgtatccatcttcccaccatccagtgagcagttaacatctggaggtgcctcagtcgtgtgcttcttgaacaacttctaccccaaagacatcaatgtcaagtggaagattgatggcagtgaacgacaaaatggcgtcctgaacagttggactgatcaggacagcaaagacagcacctacagcatgagcagcaccctcacgttgaccaaggacgagtatgaacgacataacagctatacctgtgaggccactcacaagacatcaacttcacccattgtcaagagcttcaacaggaatgagtgttag

SEQ ID NO: 183 - DNA, 336 bp, Artificial Sequence
  Description of Artificial Sequence: Synthetic polynucleotide
caggtgcagctgaaggagtcaggacctggcctggtggcgccctcacagagcctgtccatcacatgcactgtctcagggttctcattaaccagctatggtgtaagctgggttcgccagcctccaggaaagggtctggagtggctgggagtaatatggggtgacggaagcacaaattatcattcatctctcatatccagactgagcatcagcaaggataactccaagagccaagttttcttaaaactgaacagtctgcaaactgatgacacagccacgtactactgtgccagagcctttgtttactggggccaagggactctggtcactgtctctgca

SEQ ID NO: 184 - DNA, 325 bp, Artificial Sequence
  Description of Artificial Sequence: Synthetic polynucleotide
caaattgttctcacccagtctccagcaatcatgtctgcatctccaggggagaaggtcaccatgacctgcagtgccagctcaagtgtaagttacatacactggtaccagcagaagtcaggcacctcccccaaaagatggatttatgacacatccaaactggcttctggagtccctgctcgcttcagtggcagtgggtctgggacctcttactctctcacaatcagcagcatggaggctgaagatgctgccacttattactgccagcagtggagtagtaacccacccatgctcacgttcggtgctgggaccaagctggagctgaaac

SEQ ID NO: 185 - DNA, 336 bp, Artificial Sequence
  Description of Artificial Sequence: Synthetic polynucleotide
caggtgcagctgaaggagtcaggacctggcctggtggcgccctcacagagcctgtccatcacatgcactgtctcagggttctcattaaccagctatggtgtaagctgggttcgccagcctccaggaaagggtctggagtggctgggagtaatatggggtgacgggagcacaaattatcattcagctctcatatccagactgatcatcagcaaggataactccaagagccaagttttcttaaaactgaacagtctgcaaactgatgacacagccacctactactgtaccaaaggctttacttactggggccaggggactctggtcactgtctctgca

SEQ ID NO: 186 - DNA, 319 bp, Artificial Sequence
  Description of Artificial Sequence: Synthetic polynucleotide
caaattgttctcacccagtctccagcaatcatgtctgcatctccaggggagaaggtcaccatgacctgcagtgccagctcaagtgtaagttacatgcactggtaccagcagaagtcaggcacctcccccaaaagatggatttttgacacatccaaactggcttctggagtccctgctcgcttcagtggcagtgggtctgggacctcttactctctcacaatcagcagcatggaggctgaagatgctgccacttattactgccagcagtggagtagtaacctgctcacgttcggtgctgggaccaagctggagctgaaac

SEQ ID NO: 187 - DNA, 336 bp, Artificial Sequence
  Description of Artificial Sequence: Synthetic polynucleotide
caggtgcagctgcaggagtcaggacctggcctggtggcgccctcacagagcctgtccatcacatgcactgtctcagggttctcattaatcagctatggtgtaaactgggttcgccagcctccaggaaagggtctggagtggctgggagtgatatggggtgacgggagcacaaattatcagtcagctctcatatccagactgatcatcagcaaggataactccaagagccaagttttcttaaaactgaacagtctgcaaactgatgacacagccacgtactactgtaccaaaggctttgcttactggggccaagggactctggtcactgtctctgca

SEQ ID NO: 188 - DNA, 319 bp, Artificial Sequence
  Description of Artificial Sequence: Synthetic polynucleotide
caaattgttctcacccagtctccagcaatcatgtctgcatctccaggggagaaggtcaccatgacctgcagtgccagctcaagtgtaagttacatgcactggttccagcagaagtcaggcacctcccccaaaagatggatttatgacacatccaaactggcttctggagtccctgctcgcttcagtggcagtgggtctgggacctcttactctctcacaatcagcagcatggaggctgaagatgctgccacttattactgccagcagtggagtagtaacctgctcacgttcggtgctgggaccaagctggagctgaaac

SEQ ID NO: 189 - DNA, 336 bp, Artificial Sequence
  Description of Artificial Sequence: Synthetic polynucleotide
caggtgcagctgaaggagtcaggacctggcctggtggcgccctcacagaacctgtccatcacatgcactgtctcagggttctcattaaccagttatggtgtaaactgggttcgccagcctccaggaaagggtctggagtggctgggagtaatatggggtgacgggagcacaaattatcattcagctctcatttccagactgatcatcagcaaggaaaactccaagagccaagttttcttaaaactgaacagtctgcaaactaatgacacagccacgtattactgtaccaaaggctttgtttactggggccaagggactctggtcactgtctctgca

SEQ ID NO: 190 - DNA, 342 bp, Artificial Sequence
  Description of Artificial Sequence: Synthetic polynucleotide
caggtgcagctgaaggagtcaggacctggcctggtggcgccctcacagagcctgtccatcacatgcactgtctcagggttctcattaaccagctatggtgtaagctgggttcgccagcctccaggaaagggtctggagtggctgggagtaatatggggtgacgggagcacaaattatcattcagctctcatatccagactgagcatcagcaaggataactccaagagccaagttttcttaaaactgaacagtctgcaaactgatgacacagccacgtactactgtgccaaagggggctactttgactactggggccaaggcaccactctcacagtctcctca

SEQ ID NO: 191 - DNA, 319 bp, Artificial Sequence
  Description of Artificial Sequence: Synthetic polynucleotide
caaattgttctcacccagtctccagcagtcatgtctgcatctccaggggagaaggtcgccataacctgcagtgccagctcaagtgtaagttacatgcactggttccagcagaagccaggcacttctcccaaactctggatttatagcacatccaacctggcttctggagtccctgctcgcttcagtggcagtggatctgggacctcttactctctcacaatcagccgaatggaggctgaagatgctgccacttattactgccagcaaaggagtagttacccgtggacgttcggtggaggcaccaagctggaaatcaaac

SEQ ID NO: 192 - DNA, 345 bp, Artificial Sequence
  Description of Artificial Sequence: Synthetic polynucleotide
caggttcagttgctgcagtatgacgctgagttggtgaaacctggggggtcagtgaagatatcgtgcaaggcctctggctacaccttcactgaccatgctattcactgggtgaagcagaagcctgaacagggcctggaatggattggatatttttctcccggaaatgatgatattaagtacagtgagaagttcaagggcaaggccacactgactgcagacaagtcctccagcactgcctacatgcagctcaacagcctgacatctgaggattctgcagtgtatttctgtaaaagatccattactacgccttactggggccaagggactctggtcactgtctctgca

SEQ ID NO: 193 - DNA, 319 bp, Artificial Sequence
  Description of Artificial Sequence: Synthetic polynucleotide
gacatccagatgaaccagtctccatccagtctgtctgcatcccttggagacacaattaccatcacttgccatgccagtcagaacattaatgtttggttaagctggtaccagcagaaaccaggaaatattcctaaactattgatctataaggtttccaacttgcacacaggcgtcccatcaaggtttagtggcagtggatctggaacaggtttcacattaaccatcagcagcctgcagcctgaagacattgccacttactactgtcaacaggatcaaagttatccgtacacgttcggaggggggaccaagctgaaaaaaa

SEQ ID NO: 194 - DNA, 345 bp, Artificial Sequence
  Description of Artificial Sequence: Synthetic polynucleotide
caggttcagctgcagcagtctgacgctgagttggtgaaacctggggcttcagtgaagatatcctgcaaggcctctggctacaccttcactgaccatgctattcactgggtgaagcagaagcctgaacagggcctggaatggattggatatatttctcccggaaatgatgatattaagtacaatgagaagttcaagggcaaggccacactgactgcagacaaatcctccagcactgcctacatgcagctcaacagcctgacatctgaggattctgcagtgtatttctgtaaaagatccattactacgtcttactggggccaagggactctggtcactgtctctgca

SEQ ID NO: 195 - DNA, 323 bp, Artificial Sequence
  Description of Artificial Sequence: Synthetic polynucleotide
aacattgtaatgacccaatctcccaaatccatgtccatgtcagtaggagagagggtcaccttgacctgcaaggccagtgagaatgtggttatttatgtttcctggtatcaacagaaaccagagcagtctcctaaactgctgatatacggggcatccaaccggtacactggggtccccgatcgcttcacaggcagtggatctgcaacagatttcactctgaccatcagcagtgtgcaggctgaagaccttgcagattatcactgtggacagggttacagctatccgtacacgttcggaggggggaccaagctggaaataaaacg

SEQ ID NO: 196 - DNA, 345 bp, Artificial Sequence
  Description of Artificial Sequence: Synthetic polynucleotide
caggttcagttgcagcagtctgacgctgagttggtgaaacctggggcttcagtgaagatatcctgcaaggcttctggctacaccttcactgaccatgccattcattgggtgaagcagaagcctgaacagggcctggaatggattggatatgtttctcccggaaatggtgatattaagtacaatgagaagttcaagggcaaggccacactgactgcagacaaatcctccagcactgcctacatgcagctcaacagcctgacatcggaggattctgcagtgtatttctgtaaaagatctttaattggagactattggggccaaggcaccactctcacagtctcctca

SEQ ID NO: 197 - DNA, 322 bp, Artificial Sequence
  Description of Artificial Sequence: Synthetic polynucleotide
gacattgtgatgacccagtctcaaaaattcatgtcctcatcagtaggagacagggtcaccatcacctgcaaggccagtcagaatgtgggtactgctgtagcctggtatcaacagaaaccaggacaatctcctaaatttctgatttactcggcatccaatcggtacactggagtccctgatcgcttcacaggcagtggatctgggacagatttcactctcacgatcagcaatatgcagtctgaagacctggcagattatttctgccagcaatatagcagctatcgtctgacgttcggtggaggcaccaagctggaaatcaaac

SEQ ID NO: 198 - DNA, 345 bp, Artificial Sequence
  Description of Artificial Sequence: Synthetic polynucleotide
caggttcagctgcagcagtctgacgctgaattggtgaaacctggggcttcagtgaagatatcctgcaaggcttctggctacaccttcactgaccatgctattcactgggtgaagcagaagcctgaacagggcctggaatggattggatatctttctcccggaaatgatgatattaagtacagtgagaagttcaaggacaaggccacactgactgcagacaaatcctccagcactgcctacatgcagctcaacagcctgacatctgaggattctgcagtgtatttctgtaaaagatccatagggggggaccactggggccaaggcaccactctcacagtctcctca

SEQ ID NO: 199 - DNA, 323 bp, Artificial Sequence
  Description of Artificial Sequence: Synthetic polynucleotide
gacatccagatgaaccagtctccatccagtctgtctgcatcccttggagacacaattaccatcacttgccatgccagtcagaacattaatgtttggttaaactggtaccagcagaaaccaggaaatattcctaaactattgatctataaggcttccaacttgcacacaggcgtcccatcaaggtttagtggcagtggatctggaacaggtttcacattaaccatcggcagcctgcagcctgaagacattgccacttactactgtcaacagggtcaaagttatccgttcacgttcggaggggggaccaagctggaaataaaacg

SEQ ID NO: 200 - DNA, 345 bp, Artificial Sequence
  Description of Artificial Sequence: Synthetic polynucleotide
caggttcagctgcagcagtctgacgctgagttggtgaaacctggggcttcagtgaagatatcctgcaaggcttctggctacaccttcactgaccatgctattcactgggtgaaacagaagcctgaacagggcctggaatggattggatatatttctcccggaaatggtgatattaagtataatgagaagttcaagggcaaggccacactgactgcagacaaatcctccagcactgcctacatgcagctcaacagcctgacatctgaggattctgcagtgtatttctgtcaaagacaactgggacaaggctactggggccaaggcaccactctcacagtctcctca

SEQ ID NO: 201 - DNA, 338 bp, Artificial Sequence
  Description of Artificial Sequence: Synthetic polynucleotide
gatgttgtgatgacccaaactccactctccctgcctgtcagtcttggagatcaagcctccatctcttgcagatctagtcagagccttgtacacagttatggaaacacctatttacattggtacctgcagaagccaggccagtctccaaagctcctgatttacaaagtttccaaccgattttctggggtcccagacaggttcagtggcagtggatcagggacagatttcacactcaagatcagcagagtggaggctgaggatctgggagtttatttctgctctcaaaatacacatgttccgtacacgttcggaggggggaccaagctggaaataaaacg

SEQ ID NO: 202 - DNA, 345 bp, Artificial Sequence
  Description of Artificial Sequence: Synthetic polynucleotide
caggttcagctgcagcagtctgacgctgagttggggaaacctggggcttcagtgaagatatcctgcaaggcttctggctacaccttcagtgaccatgctattcactgggtgaagcagaagcctgaacagggcctggaatggattggatatatctctcccggaaacgatgatattaagtacaatgagaagttcaagggcaaggccacactgactgcagacaaatcctccagcactgcctacatgcagctcaacagcctgacatctgaggattctgcagtgtatttctgtgaaagatcgatgattggggtttactggggccaagggactctggtcactgtctctgca

SEQ ID NO: 203 - DNA, 337 bp, Artificial Sequence
  Description of Artificial Sequence: Synthetic polynucleotide
gatgttgtgatgacccaaactccactctccctgactgtcagtcttggcgatcaagcctccatctcttgcagatttagtcagagccttgtacaaagtaatggaaatacctatttacagtggtatctgcagaagccaggccagtctccaaagctcctgatttacaaagtctccaaccgattttgtggggtcccagacaggttcagtggcagtggatcagggacagatttcacactcaagatcagcagagtggaggctgaggatctgggagtttatttctgctctcaaagtacacatgctccgctcacgttcggtgctgggaccaagctggagctgaaac

SEQ ID NO: 204 - DNA, 342 bp, Artificial Sequence
  Description of Artificial Sequence: Synthetic polynucleotide
caggttcagctgcagcagtctgacgctgagttggtgaaacctggggcttcagtgaagatatcctgcaagacttctggctacaccttcactgaccatgcaattcactgggtgaagcagaagcctgaacagggcctggaatggattggatatatttctcccggaaatggtgatattaagtacaatgagaagttcaagggcaaggccaccctgactgcagacaaatcctccagcactgcctatatgcagctcagcagcctgacacctgaggattctgcagtgtatttctgtaaaatatcttactacggtatttggggccaaggcaccactctcacagtctcctca

SEQ ID NO: 205 - DNA, 322 bp, Artificial Sequence
  Description of Artificial Sequence: Synthetic polynucleotide
gacatccagatgactcagtctccagcctccctatctgtatctgtgggagagtctgtcaccatcacatgtcgactaagtgaagatatttacagtaatttagcatggtttcagcagagaccgggaaaatctcctcagctcctggtttataaagcaacaaacttagcagacggtgtgccatcaaggttcagtggcagtggatcaggcacacagtattccctcaagatcaacagcctgcagtctgaagattttgggacttattactgtcaacatttttggggtactccattcacgttcggctcggggaccaaggtggaaataaaac

SEQ ID NO: 206 - DNA, 342 bp, Artificial Sequence
  Description of Artificial Sequence: Synthetic polynucleotide
caggttcagctgcagcagtctgacgctgagttggtgaaacctggggcttcagtgaagatatcctgcaaggcttctggctacaccttcactgaccatgctattcactgggtgaagcagaagcctgaacagggcctggaatggattggatatttttctcccggaaatgatgatattaagtataatgagaagttcaaggtcaaggccacactgactgcagacaaatcctccagcactgcctacatgcaactcaccagcctgacatctgaagattctgcagtgtatttctgtaaaagatcttactacggtgattggggccaaggcaccactctcacagtctcctca

SEQ ID NO: 207 - DNA, 322 bp, Artificial Sequence
  Description of Artificial Sequence: Synthetic polynucleotide
gacatccagatgactcagtctccagcctccctatctgtttctgtgggagaaactgtcaccatcacatgtcgagcaagtgagaatatttacagtcatttagcatggtatcaacagaaacagggaaaatctcctcaactcctggtctatggtgcaactaacttagcagatggtgtgccatcaaggttcagtggcagtggatcaggcacacagttttccctcaagatccacagcctgcagtctgaagattttgggagttattactgtcaacatttttggggtgctccattcacgttcggctcggggacaaagttggaaataaaac

SEQ ID NO: 208 - DNA, 345 bp, Artificial Sequence
  Description of Artificial Sequence: Synthetic polynucleotide
caaattcagctgcagcagtctgacgctgagttggtgaaacctgggacttcagtgaagatgtcctgcaaggcttctggctacaccttcactgaccatgctattcactgggtgaagcagaagcctgaacagggcctggaatggattggatatttttctcccggaaatgatgatattaagtataatgtgaagttcaagggcaaggccacactgactgcagacaaatcctccagcactgcctacatgcagctcaacagcctgacatctgaagattctgcagtgtatttctgttcggtgggatacgcccttgactactggggcctaggcaccactctcacagtctcctca

SEQ ID NO: 209 - DNA, 323 bp, Artificial Sequence
  Description of Artificial Sequence: Synthetic polynucleotide
aacattgtaatgacccaatctcccaaatccatgtccatgtcagtaggagagagggtcaccttgacctgcaaggccagtgagaatgtggttacttatgtttcctggtatcaacagaaaccagagcagtctcctaaactgctgatatacggggcatccaaccggtacactggggtccccgatcgcttcacaggcagtggatctgcaacagatttcactctgaccatcagcagtgtgcaggctgaagaccttgcagattatcactgtggacagggttacagctatccgtacacgttcggaggggggaccaagctggaaataaaacg

SEQ ID NO: 210 - DNA, 345 bp, Artificial Sequence
  Description of Artificial Sequence: Synthetic polynucleotide
caggttcagctgcaacagtctgacgctgagttggtgaaacctgggactacagtgaagatatcctgcaaggcttctggctacactttcactgaccatgctattcactgggtgaaggagaagcctgaacagggcctggaatggatcggatatatttctcccggaaatgatgatattaagtacagtgagaagttcaagggcaaggccacactgactgcagacaaatcctccagcactgcttacatgcagctcaacagcctgacatctgatgattctgcagtgtatttctgtaaaagatcgcttagtacgccttactggggccaagggactctggtcactgtctctgca

SEQ ID NO: 211 - DNA, 477 bp, Artificial Sequence
  Description of Artificial Sequence: Synthetic polynucleotide
tttttaatacgactccctatagggcaagcagtggtatcaatgcagattacaagggggaaaggcatcagaccagcatgggcatcaaggtggaatcacagactctggtcttcatatccatactgtttgggttatatggagctgatgggaacacattaatgacccaatctcccacatccatgtacatgtcagtaggagagagggtcaccttgacttgcaaggccagtgagaatgagattaattatgtttcctggtatcaacagaaaccagagcagtctcctaaactgttgatatacggggcatccaaccggtactctggggtccccgatcgcttcacaggcagtggatctgcaacagatttcactctgaccatcagcagtgtgcaggctgaagaccttgcagattatccctgtggagcaagggattaactagctatccgtacacgttcggaggggggaccaagctggaaataaaacgggc

SEQ ID NO: 212 - DNA, 341 bp, Artificial Sequence
  Description of Artificial Sequence: Synthetic polynucleotide
gacattgtgatgacacagtctccatcctccctgactgtgacagcaggagagaaggtcactatgagctgcaggtccagtcagagtctgttaaacagtggaaatcaaaagaactacttgacctggtaccagcagaaaccagggcagcctcctaaactgttgatctactgggcatccactagggaatctggggtccctgatcgcttcacaggcagtggatctggaacagatttcactctcaccatcagcagtgtgcaggctgaagacctggcagtttattactgtcagaatgattatagttatccgtacacgttcggaggggggaccaagctggaaataaaacg

SEQ ID NO: 213 - DNA, 343 bp, Artificial Sequence
  Description of Artificial Sequence: Synthetic polynucleotide
caggttcagctgcagcagtctgacgctgagttggtgaaacctggggcttcagtgaagatatcctgcaaggcttctggctacaccttcactgaccatgctattcactgggtgatgcagatgcctgaacagggcctggaatggattggatatatttctcccggaaatggtgatgttaagtacagtgagaggttcaagggcagggccacactgactgcagacaaatcctccagctctgcctacatgcagctcaacagcctgacatctgaggattctgcagtttatttctgtaaaagatcgcttagtacgccttactggggccaagggactctggtcactgtctctg

SEQ ID NO: 214 - DNA, 341 bp, Artificial Sequence
  Description of Artificial Sequence: Synthetic polynucleotide
gacattgtgatgacacagtctccatcctccctgactgtgacagcaggagagagggtcactatgagctgcaagtccagtcagagtctgttaaacagtggaaatcaaaagagctacttgacctggtaccagcagaaaccagggcagcctcctaaactgttgatctcctgggcatccactagggattctggggtccctgatcgcttcacaggcagtggatctggaacagatttcactctcaccatcagcagtgtgcaggctgaagacctggcagtttattactgtcagagtgattatagttatccgtacacgttcggaggggggaccaagctggaaataaaacg

SEQ ID NO: 215 - DNA, 345 bp, Artificial Sequence
  Description of Artificial Sequence: Synthetic polynucleotide
  modified_base (26)..(26): a, c, g, t or not present
  modified_base (332)..(332): a, c, g, t or not present
caggttcagctgcagcagtctgacgntgagttggtgaaaccgggggcttcagtgaagatatcctgtaaggcttctggctacaccttcactgaccatgctattcactgggtgaagcagaagcctgaacagggcctggaatggattggatatttttctcccggaaatgatgatattaagtacaatgagaagtttaggggcaaggccacactgactgcagacaaatcctccagcactgcctacatgcagctcaacagcctgtcatctgatgattctgcagtgtatttctgtaaaagatcgcttagtacgccttactggggccaagggactctggncactgtctctgca

SEQ ID NO: 216 - DNA, 341 bp, Artificial Sequence
  Description of Artificial Sequence: Synthetic polynucleotide
gacattgtgatgacacagtctccatcctccctgactgtgacagcaggagagaaagtcactatgagctgcaagtccagtcagagtctgttaaaccgtggaaatcataagaactacttgacctggtaccggcagaaaccagggctgcctcctaaactgttgatttactgggcatccactagggaatctggggtccctgatcgcttcacaggcagtggatctggaacagatttcgctctcaccatcagcagtgttcaggctgaagacctggcagtttattactgtcagaatgattatacttatccgtacacgttcggaggggggaccaagctggagataaaacg

SEQ ID NO: 217 - DNA, 345 bp, Artificial Sequence
  Description of Artificial Sequence: Synthetic polynucleotide
caggttcagctgcagcagtctgacgctgagttggtgaaacctggggcttcaatgaagatttcctgcaaggcttctggctacaccttcactgaccatgctattcactgggtgaagcagaagcctgaacagggcctggaatggattggatatatttctcccggaaatggtgatattaagtacaatgagaagttcaaggtcaaggccacactgactgcagacaaatcctccagcactgcctacatgcagctcaacagcctgacatctgaggattctgcagtgtatttctgtaaaagatcgattactacgccttactggggccaagggactctggtcactgtctctgca

SEQ ID NO: 218 - DNA, 341 bp, Artificial Sequence
  Description of Artificial Sequence: Synthetic polynucleotide
gacattgtgatgacacagtctccatcctccctgactgtgacagcaggagagaaggtcactatgagctgcaagtccagtcagagtctgttaaacagtggaaaaacaaagaactacttgacgtggtaccagcagaaaccagggcagcctcctaaactgttgatctactgggcatccactagggaatctggggtccctgatcgcttcacaggcagtggatctggaacagatttcactctcaccatcagcagtgtgcaggctgaagacctggcagtttattactgtaagaatgattatagttatccgtacacgttcggaggggggaccaagctggaaataaaacg

SEQ ID NO: 219 - DNA, 345 bp, Artificial Sequence
  Description of Artificial Sequence: Synthetic polynucleotide
caggttcagctgcagcagtctgacgctgaattggtgaagcctggggcttcagtgaagatatcctgcaagacttctggctacaccttcactgaccatgctattcactgggtgaagcagaagcctgaacagggcctggaatggattggatatatctctcccggaaatgatgatattaagtacactgagaagttcaagggcaaggtcacactgactgcagacaaatcctccagcactgcctacatgcagctcaacagcctgacatctgaggattctgcagtctatttctgtaaaagatcgattactacgccttactggggccaagggactctggtcactgtctctgca

SEQ ID NO: 220 - DNA, 480 bp, Artificial Sequence
  Description of Artificial Sequence: Synthetic polynucleotide
  modified_base (153)..(153): a, c, g, t or not present
  modified_base (285)..(286): a, c, g, t or not present
  modified_base (289)..(289): a, c, g, t or not present
  modified_base (297)..(298): a, c, g, t or not present
  modified_base (332)..(332): a, c, g, t or not present
  modified_base (405)..(405): a, c, g, t or not present
  modified_base (412)..(412): a, c, g, t or not present
  modified_base (429)..(429): a, c, g, t or not present
tttttatacgccactttctaatacgcctcactatagggcaagcagtggtatcaacgcagattacaaaggggaaaggaatcagaccgactcgcgcatcaagatggaatcacagactctggtcttcatatccagtacgctcggggactatggagnggaacagtacattttaatgacccaatgtcccaaaggcaagaacatgtcagtaggagagagggtcactcagagtgcaaggccaggagaaatcaaaacacttatgtttcctggtatcaacagaaaccagagcannctntaaaatgnngattacggggcatccaaccgggaatctggggtcnccgatcgcttcacaggcagtggatctggaacagatttcactctcaccatcagcagtgtgcaggctgaagaccnggcagtnttcactgtggacagggntacagttatccgtacacgttcggaggggggaccaagctgaaaaaaacgggc

SEQ ID NO: 221 - DNA, 345 bp, Artificial Sequence
  Description of Artificial Sequence: Synthetic polynucleotide
caggttcagctgcagcagtctgacgctgagttggtgaaacctggggcttcagtgaagatatcctgcaaggcttctggctacaccttcactgaccatgctattcactgggtgaagcagaagcctgaacagggcctggaatggattggatatatttctcccggaaatggtgatattaagtacgatgagaagtttaagggcaaggccacactgactgcagacaaatcctcctccactgcctacatgcagctcaacagcctgacatctgaagattctgcagtgtatttctgtaaaagatcgattactacctcttactggggccaagggactctggtcactgtctctgca

SEQ ID NO: 222 - DNA, 345 bp, Artificial Sequence
  Description of Artificial Sequence: Synthetic polynucleotide
caggttcagctgcagcagtctgacgctgagttggtgaaacctggggcttcagtgaagatatcctgcaaggcttctggctacaccttcactgaccatgctattcactgggtgaagcagaagcctgaacagggcctggaatggattggatatatttctcccggaaatgatgatattaagtacaatgagaagttcaagggcaaggccacactgactgcagacaagtcctccagcactgcctacatgcagctcaacagcctgacatctgaggattctgcagtgtttttctgtaaaagatcgattactacctcttactggggccaagggactctggtcactgtctctgca

SEQ ID NO: 223 - DNA, 483 bp, Artificial Sequence
  Description of Artificial Sequence: Synthetic polynucleotide
  modified_base (3)..(3): a, c, g, t or not present
  modified_base (137)..(137): a, c, g, t or not present
  modified_base (193)..(193): a, c, g, t or not present
ttnataggactcaatatagggcaagcagtggtattaacgccgagtacatggggagggcaagggcagaaagtcactttcagtgaggatacaccatcagcatgagggtccttgttgagctcctgggggggctggtgttntgctttttaggtgtgagatgtgacatccagatgaaccagtctccatccagtctgtntgcatcctttggagacacaattaccatcatttgccattccagtcagaacattaatgtttggttaagatggtaccagcagaaaccaggaaatattcctaaaatattgatatataagggttccaacttgtacacaggcgtcccatcaaggtttagtggcagtggatttggaacaggtttcacattaaccatcagcagcgtgcagcgggaagacattgccacttactactgtcaacaggatcaaagttatccgtacacgttcggaggggggaccaagctgaaataaaacgggc

SEQ ID NO: 224 - DNA, 345 bp, Artificial Sequence
  Description of Artificial Sequence: Synthetic polynucleotide
caggttcagctgcagcagtctgacgccgagttggtgaaacctggggcttcagtgaagatatcctgcaaggcttctggctacatcttcactgaccatgctattcactgggtgaagcagaagcctgaacagggcctggaatggattggatatatttctcccggaaatggtgatattaagtacaatgagaagttcaagggcaaggccacactgactgcagacaaatcctccagcactgcctacatgcatctcaacagcctgacatctgaggattctgcagtgtatttctgtaaaagatcgattactacctcttactggggccaagggactctggtcactgtctctgca

SEQ ID NO: 225 - DNA, 323 bp, Artificial Sequence
  Description of Artificial Sequence: Synthetic polynucleotide
gacatccagatgaaccagtccccatccagtctgtctgcatcccttggagacacaattaccatcacttgccatgccagtcagcacattaatttttggttaagctggtaccagcagaaaccaggaaatattcctaaactcttgatctataaggcttccaacttgcacacaggcgtcccatcaaggtttagtggcagtggatctggaacaggtttcacattaaccatcagcagcctgctgcctgaagacgttgccacttactactgtcaacaggatcaaagttatccgtatatgttcggaggggggaccaagctggaaataaaacg

SEQ ID NO: 226 - DNA, 345 bp, Artificial Sequence
  Description of Artificial Sequence: Synthetic polynucleotide
caggttcagctgcagcagtctgacgctgagttggtgaaacctggggcttcagtgaagatatcctgcaaggcttctggctacaccttcactgaccatgctattcactgggtgaagcagaagcctgaacagggcctggaatggattggatatatttctcccggaaatgatgatattaagtacaatgagaagtttaagggcaaggccacactgactgcagacaaatcctccagcactgcctacatgctgctcaacagcctgacatctgaggattctgcagtgtatttctgtaaaagatcgattactacctcttactggggccaagggactctggtcactgtctctgca

SEQ ID NO: 227 - DNA, 323 bp, Artificial Sequence
  Description of Artificial Sequence: Synthetic polynucleotide
aacattgtaatgacccaatctcccaaatccatgtccatgtcagtaggagagagggtcaccttgacctgcaaggccagtgagaatgtggttacttatgtttcctggtatcaacagaaaccagagcagtctcctaaactgctgatatacggggcatccaaccggtacactggggtccccgatcgcttcacaggcagtggatctgcaacagatttcactttgaccatcagcagtgtgcaggctgaagaccttgcagattatcactgtggacagggttacagctatccgtacacgttcggaggggggaccaagctggaaataaaacg

SEQ ID NO: 228 - DNA, 345 bp, Artificial Sequence
  Description of Artificial Sequence: Synthetic polynucleotide
caggttcaactgcagcagtctgacgctgagttggtgaaacctggggcttcagtgaagatatcctgcaaggcttctggctacaccttcactgaccatgctattcactgggtgaagcagaagcctgaacagggcctggaatggattggatatatttctcccggaaatggtgatattaagtacaatgagaagttcaagggtaaggccacactgactgcagacacttcctccaccactgcctacatgcagctcaacagcctgacatctgaggattctgcaatgtatttctgtaaaagatccattactacgtcttactggggccaagggactctggtcactgtctctgca

SEQ ID NO: 229 - DNA, 345 bp, Artificial Sequence
  Description of Artificial Sequence: Synthetic polynucleotide
caggttcagctgcagcagtctgacgctgagttggtgaaacctggggcttcagtgaagatatcctgcaaggcttctggctacatcttcactgaccatgcaattcactgggtgaagcagaagcctgaacagggcctggaatggattggatatatttctcccggaaatggtgatattaagtacattgagaagttcaggggcaaggccacactgactgcagacaaatcctccagcactgcctacatgcagctcaacagcctgacatctgaggattctgcagtgtatttctgtaaaagatcgcttagtacgccttactggggccaagggactctggtcactgtctctgca

SEQ ID NO: 230 - DNA, 329 bp, Artificial Sequence
  Description of Artificial Sequence: Synthetic polynucleotide
aacattttaatgacccaatctcccaaatccatgtccatgtcagtaggagagagggtcaccttgacctgcaaggccagtgagaatgtggttaattatgtttcctggtatcaacagaaaccagagcagtctcctaaactgctgatattcggggcatccaaccggtactctggggtccccgatcgcttcacaggcagtggatctgcaacagatttcactctgaccatcagcagtgtgcaggctgaagaccttgcagattatcactgtggaagcaagtggattactagctatccgtacacgttcggaggggggaccaagctggaaataaaacg

SEQ ID NO: 231 - DNA, 326 bp, Artificial Sequence
  Description of Artificial Sequence: Synthetic polynucleotide
aacattttaatgacccaatctcccaaatccatgtccatgtcagtaggagagagggtcaccttgacctgcaaggccagtgagaatgtggttaattatgtttcctggtatcaacagaaaccagagcagtctcctaaactgctgatatacggggcatccaaccggtactctggggtccccgatcgcttcacaggcagtggatctgcaacagatttcactctgaccatcagcagtgtgcaggctgaagaccttgcagattatcactgtggagcaagggttactagctatccgtacacgttcggaggggggaccaagctggaaataaaacg

SEQ ID NO: 232 - DNA, 345 bp, Artificial Sequence
  Description of Artificial Sequence: Synthetic polynucleotide
caggttcagctgcagcagtctgacgctgagttggtgaaacctgggacttcagtgaagatatcctgcagggcttctggctacaccttcactgaccatgctattcactgggtgaagcagaagcctgaacagggcctggaatggattggatatatttctcccggaaatggtgatattaagtacaatgagaagttcaagggcaaggccacactgactgcagacaaatcctccagcactgcctacatgcagctcaacagcctgacatctgacgattctgcagtgtatttctgtaaaagatccattactacgccttactggggccaaggcaccactctcacagtctcctca

SEQ ID NO: 233 - DNA, 315 bp, Artificial Sequence
  Description of Artificial Sequence: Synthetic polynucleotide
agttttgtgatgacccagactcccaaattcctgcttgtgtcagcaggagacagggttaccataacctgcaaggccagtcagagtgtgaataataatgtagcttggtaccaacagaagccagggcagtctcctaaacagctgatatactatgcatccaatcgctacactggagtccctgatcgcttcactggcagtggatatgggacggatttcactttcaccatctacactgtgcaggctgaagacctggcagtttatttctgtcagcagggttatagctctccgtggacgttcggtggaggcaccaagctgaaa

SEQ ID NO: 234 - protein, 330 aa, Artificial Sequence
  Description of Artificial Sequence: Synthetic polypeptide
AKTTAPSVYPLAPVCGDTTGSSVTLGCLVKGYFPEPVTLTWNSGSLSSGVHTFPAVLQSDLYTLSSSVTVTSSTWPSQSITCNVAHPASSTKVDKKIEPRGPTIKPCPPCKCPAPNLLGGPSVFIFPPKIKDVLMISLSPIVTCVVVDVSEDDPDVQISWFVNNVEVHTAQTQTHREDYNSTLRVVSALPIQHQDWMSGKEFKCKVNNKDLPAPIERTISKPKGSVRAPQVYVLPPPEEEMTKKQVTLTCMVTDFMPEDIYVEWTNNGKTELNYKNTEPVLDSDGSYFMYSKLRVEKKNWVERNSYSCSVVHEGLHNHHTTKSFSRTPGK

SEQ ID NO: 235 - protein, 107 aa, Artificial Sequence
  Description of Artificial Sequence: Synthetic polypeptide
RADAAPTVSIFPPSSEQLTSGGASVVCFLNNFYPKDINVKWKIDGSERQNGVLNSWTDQDSKDSTYSMSSTLTLTKDEYERHNSYTCEATHKTSTSPIVKSFNRNEC

SEQ ID NO: 236 - protein, 446 aa, Artificial Sequence
  Description of Artificial Sequence: Synthetic polypeptide
QVQLQQSDAELVKPGASVKISCKASGYTFTDHAIHWVKQKPEQGLDWIGYISPGNGDIKYNEKFKDKVTLTADKSSSTACMHLNSLTSEDSAVYFCKRSLLALDYWGQGTTLTVSSAKTTAPSVYPLAPVCGDTTGSSVTLGCLVKGYFPEPVTLTWNSGSLSSGVHTFPAVLQSDLYTLSSSVTVTSSTWPSQSITCNVAHPASSTKVDKKIEPRGPTIKPCPPCKCPAPNLLGGPSVFIFPPKIKDVLMISLSPIVTCVVVDVSEDDPDVQISWFVNNVEVHTAQTQTHREDYNSTLRVVSALPIQHQDWMSGKEFKCKVNNKDLPAPIERTISKPKGSVRAPQVYVLPPPEEEMTKKQVTLTCMVTDFMPEDIYVEWTNNGKTELNYKNTEPVLDSDGSYFMYSKLRVEKKNWVERNSYSCSVVHEGLHNHHTTKSFSRTPGK

SEQ ID NO: 237 - DNA, 1401 bp, Artificial Sequence
  Description of Artificial Sequence: Synthetic polynucleotide
atggagaccgacaccctgctgctctgggtgctgctgctctgggtgcccggctccaccggacaggttcagctgcagcagtctgacgctgagttggtgaaacctggggcttcagtgaagatatcctgcaaggcttctggctacaccttcactgaccatgctattcactgggtgaagcaaaagcctgaacagggcctggactggattggatatatttctcccggaaatggtgatattaagtacaatgagaagttcaaggacaaggtcacactgactgcagacaaatcctccagcactgcctgcatgcacctcaacagcctgacatctgaggattctgcagtgtatttctgcaaaagatccctactagctcttgactactggggccaaggcaccactctcacagtctcctcagctaaaacaacagccccatcggtctatccactggcccctgtgtgtggagatacaactggctcctcggtgactctaggatgcctggtcaagggttatttccctgagccagtgaccttgacctggaactctggttccctgtccagtggtgtgcacaccttcccagctgtcctgcagtctgacctctacaccctcagctcaagcgtgactgtaaccagctcgacctggcccagccagtccatcacctgcaatgtggcccacccggcaagcagcaccaaggtggacaagaaaattgagcccagagggcccacaatcaagccctgtcctccatgcaaatgcccagcacctaacctcttgggtggaccatccgtcttcatcttccctccaaagatcaaggatgtactcatgatctccctgagccccatagtcacatgtgtagtcgttgatgtgagcgaggatgacccagatgtccagatcagctggtttgtgaacaacgtggaagtgcacactgctcagacacagacgcatagagaggattacaacagtactctccgggttgtcagtgccctccccatccagcaccaggactggatgagtggcaaggagttcaaatgcaaggtcaacaacaaagacctcccagcgcccatcgagagaaccatctcaaaacccaaagggtcagtaagagctccacaggtatatgtcttgcctccaccagaagaggagatgactaagaaacaggtcactctgacctgcatggtcacagacttcatgcctgaagacatttacgtggagtggaccaacaacgggaaaacagagctaaactacaagaacactgaaccagtcctggactctgatggttcttacttcatgtacagcaagctgagagtggagaagaagaactgggtggagagaaatagctactcctgttcagtggtccacgagggtctgcacaatcaccacacgactaagagcttctcccggactccgggtaaatag

SEQ ID NO: 238 - protein, 214 aa, Artificial Sequence
  Description of Artificial Sequence: Synthetic polypeptide
DIVMTQSHKFMSTSVGDRVSITCKASQDVGTNIAWYQQKPGRSPKVLIYSASTRHTGVPDRFTGSGSGTDFTLTISNVQSEDLTDYFCQQYSSFPLTFGVGTKLELKRADAAPTVSIFPPSSEQLTSGGASVVCFLNNFYPKDINVKWKIDGSERQNGVLNSWTDQDSKDSTYSMSSTLTLTKDEYERHNSYTCEATHKTSTSPIVKSFNRNEC

SEQ ID NO: 239 - DNA, 705 bp, Artificial Sequence
  Description of Artificial Sequence: Synthetic polynucleotide
atggagaccgacaccctgctgctctgggtgctgctgctctgggtgcccggctccaccggagacattgtgatgacccagtctcacaaattcatgtccacatcagtaggagacagggtcagcatcacctgcaaggccagtcaggatgtgggcactaatatagcctggtatcaacagaaaccaggccgatctcctaaagtactgatttactcggcatccacccggcacactggagtccctgatcgcttcacaggcagtggatctgggacagatttcactctcaccattagcaatgtgcagtctgaagacttgacagattatttctgtcagcaatatagcagctttcctctcacgttcggtgttgggaccaagctggagctgaaacgggcagatgctgcaccaactgtatccatcttcccaccatccagtgagcagttaacatctggaggtgcctcagtcgtgtgcttcttgaacaacttctaccccaaagacatcaatgtcaagtggaagattgatggcagtgaacgacaaaatggcgtcctgaacagttggactgatcaggacagcaaagacagcacctacagcatgagcagcaccctcacgttgaccaaggacgagtatgaacgacataacagctatacctgtgaggccactcacaagacatcaacttcacccattgtcaagagcttcaacaggaatgagtgttga

SEQ ID NO: 240 - protein, 12 aa, Artificial Sequence
  Description of Artificial Sequence: Synthetic peptide
CQFDLSTRRLKC

SEQ ID NO: 241 - protein, 12 aa, Artificial Sequence
  Description of Artificial Sequence: Synthetic peptide
CQYNLSSRALKC

SEQ ID NO: 242 - protein, 4 aa, Artificial Sequence
  Description of Artificial Sequence: Synthetic peptide
KDEL

SEQ ID NO: 243 - protein, 10 aa, Artificial Sequence
  Description of Artificial Sequence: Synthetic peptide
EQKLISEEDL

SEQ ID NO: 244 - protein, 8 aa, Artificial Sequence
  Description of Artificial Sequence: Synthetic peptide
DYKDDDDK